European Patent Specification EP 4 125 971 B1, published March 4, 2026. Title: Bacterial strains, the compositions thereof and use thereof in a method for the treatment of vitamin D deficiency, and disorders associated therewith. Applicant: SOFAR S.P.A. The sequence listing filed with the application follows.

SEQUENCE LISTING (2 sequences)

SEQ ID NO: 1 - DNA, 18 bp, Artificial Sequence
  Vitamin D receptor VDR hVDR Primer F
ggactgccgcatcaccaa

SEQ ID NO: 2 - DNA, 18 bp, Artificial Sequence
  Vitamin D receptor VDR hVDR Primer R
tcatctcccgcttcctct